European Patent Application EP 4 603 601 A1, published August 20, 2025. Title: Semi-dominant Molecular Marker Related to Maize Dwarf and Application thereof. Applicant: Anhui Agricultural University. The sequence listing filed with the application follows.

SEQUENCE LISTING (5 sequences)

SEQ ID NO: 1 - DNA, 1878 bp, Zea mays
  source 1..1878: mol_type = genomic DNA
atgaagcgcgagtaccaaaacgccggcgggaacgacggctacaggggctcctccaaggacaagtcgatggcggcggcggcgggggcaggggagcaggaggaggaggtggacgagctgctggcggcgctcgggtacaaggtgcgttcgtcggatatggcggacgtcgcgcagaagctagagcagctcgagatggccatggggatgggcggcgcctgccccaccgctgatgacgggttcgtctcgcacctcgccacggacaccgtgcactacaatccctccgacctgtcgtcctgggtcgagagcatgctgtccgagctcaacgcgcccccgccgccgctcccacccgcgacgccggcaccaaggctggcgtccacctcgtccaccgtcacaagtggcgccgccgccggtgccggctacttcgatctcccgcccgccgtcgactcgtccagcagtacctacgctctgaagccgatcccctcgccggtggcggcggcgtcggccgacccgtccccggactcggcgcgggagcccaagcggatgcgaactggcggcggcagcacgtcgtcgtcctcttcctcgtcgtcatccatggacggcggccgcactaggagctccgtggtcgaagctgccccgccggcgacgcaggcggccaacgggccggcggtgccggtggtggtggtggacacgcaggaggccgggatccggctggtgcacgcgctgctggcgtgcgcggaggccgtgcagcaggagaacttctctgcggcggacgcgctggtgaagcagatccccgtgctggcctcgtcgcagggcggcgccatgcgcaaggtcgccgcctacttcggcgaggcgctcgcccggcgcgtgtatcgcctccgcccggcaccggacggctccctcctcgacgccgccttcgccgacctcctgcacgcgcacttctacgagtcctgcccctacctcaagttcgcccacttcaccgcgaaccaggccatcctcgaggctttcgccgggtgccgccgcgtccacgtcgtcgacttcggcatcaagcaggggatgcagtggccggctctcctccaggccctcgccctccgccccggcggccccccgtcgttccgtctcaccggcgtaggcccgccgcagcccgacgagaccgacgccctgcagcaggtgggctggaagctcgcccagttcgcgcacaccatccgcgtcgacttccagtaccgtggcctcgtcgccgccacgctcgctgacctggagccgttcatgctgcgaccggagggcggcggcgacacggacgacgagcccgaggtgatcgccgtaaactcggtgtgcgagctgcaccggctgctcgcgcagcccggtacactcgacaaggtcctgggcaccgtgcgcgcggtgcggccgaggatcgtgacggtggtggagcaggaggccaaccacaactccggcacattcctcgaccgcttcacggagtcgctgcactactactccaccatgttcgactccctcgagggcgccggctcaggctccggctccggctccggctccggccagcccaccgacgcctccccgccggccggcacggaccaggtgatgtccgaggtgtacctcggccggcagatctgcaacatcgtggcgtgcgagggcgccgagcgcacggagcgccacgagacgctggtccagtggcgcggccgcctcggcgggtccgggttcgagcccgtgcacctgggatccaacgcctacaagcaggcaagcacgctgctggccctcttcgccggcggcgacgggtacagggtggaggagaaggacgggtgcctgactctgggatggcatacgcgcccgctcatcgccacctcggcgtggcgcgtcgccgctccgtga

SEQ ID NO: 2 - DNA, 1878 bp, Zea mays
  source 1..1878: mol_type = genomic DNA
atgaagcgcgagtaccaaaacgccggcgggaacgacggctacaggggctcctccaaggacaagtcgatggcggcggcggcgggggcaggggagcaggaggaggaggtggacgagctgctggcggcgctcaggtacaaggtgcgttcgtcggatatggcggacgtcgcgcagaagctagagcagctcgagatggccatggggatgggcggcgcctgccccaccgctgatgacgggttcgtctcgcacctcgccacggacaccgtgcactacaatccctccgacctgtcgtcctgggtcgagagcatgctgtccgagctcaacgcgcccccgccgccgctcccacccgcgacgccggcaccaaggctggcgtccacctcgtccaccgtcacaagtggcgccgccgccggtgccggctacttcgatctcccgcccgccgtcgactcgtccagcagtacctacgctctgaagccgatcccctcgccggtggcggcggcgtcggccgacccgtccccggactcggcgcgggagcccaagcggatgcgaactggcggcggcagcacgtcgtcgtcctcttcctcgtcgtcatccatggacggcggccgcactaggagctccgtggtcgaagctgccccgccggcgacgcaggcggccaacgggccggcggtgccggtggtggtggtggacacgcaggaggccgggatccggctggtgcacgcgctgctggcgtgcgcggaggccgtgcagcaggagaacttctctgcggcggacgcgctggtgaagcagatccccgtgctggcctcgtcgcagggcggcgccatgcgcaaggtcgccgcctacttcggcgaggcgctcgcccggcgcgtgtatcgcctccgcccggcaccggacggctccctcctcgacgccgccttcgccgacctcctgcacgcgcacttctacgagtcctgcccctacctcaagttcgcccacttcaccgcgaaccaggccatcctcgaggctttcgccgggtgccgccgcgtccacgtcgtcgacttcggcatcaagcaggggatgcagtggccggctctcctccaggccctcgccctccgccccggcggccccccgtcgttccgtctcaccggcgtaggcccgccgcagcccgacgagaccgacgccctgcagcaggtgggctggaagctcgcccagttcgcgcacaccatccgcgtcgacttccagtaccgtggcctcgtcgccgccacgctcgctgacctggagccgttcatgctgcgaccggagggcggcggcgacacggacgacgagcccgaggtgatcgccgtaaactcggtgtgcgagctgcaccggctgctcgcgcagcccggtacactcgacaaggtcctgggcaccgtgcgcgcggtgcggccgaggatcgtgacggtggtggagcaggaggccaaccacaactccggcacattcctcgaccgcttcacggagtcgctgcactactactccaccatgttcgactccctcgagggcgccggctcaggctccggctccggctccggctccggccagcccaccgacgcctccccgccggccggcacggaccaggtgatgtccgaggtgtacctcggccggcagatctgcaacatcgtggcgtgcgagggcgccgagcgcacggagcgccacgagacgctggtccagtggcgcggccgcctcggcgggtccgggttcgagcccgtgcacctgggatccaacgcctacaagcaggcaagcacgctgctggccctcttcgccggcggcgacgggtacagggtggaggagaaggacgggtgcctgactctgggatggcatacgcgcccgctcatcgccacctcggcgtggcgcgtcgccgctccgtga

SEQ ID NO: 3 - DNA, 439 bp, Zea mays
  source 1..439: mol_type = genomic DNA
gagctcggacagcatgctctcgacccaggacgacaggtcggagggattgtagtgcacggtgtccgtggcgaggtgcgagacgaacccgtcatcagcggtggggcaggcgccgcccatccccatggccatctcgagctgctctagcttctgcgcgacgtccgccatatccgacgaacgcaccttgtacccgagcgccgccagcagctcgtccacctcctcctcctgctcccctgcccccgccgccgccgccatcgacttgtccttggaggagcccctgtagccgtcgttcccgccggcgttttggtactcgcgcttcatgatctcggagctacaggccgggctagccagctaataattgcttgcgcccctccgtatcggttccgggatagcttgggatttggatccagggttgggaattgggagttgggaaggaaacgga

SEQ ID NO: 4 - DNA, 20 bp, Artificial Sequence
  source 1..20: mol_type = genomic DNA
gagctcggacagcatgctct

SEQ ID NO: 5 - DNA, 24 bp, Artificial Sequence
  source 1..24: mol_type = genomic DNA
tccgtttccttcccaactcccaat